European Patent Application EP 4 215 624 A1, published July 26, 2023. Title: Method and Kit for Multiple Detection of Respiratory Virus Nucleic Acid. Applicant: Daan Gene Co., Ltd. The sequence listing filed with the application follows.

SEQUENCE LISTING (21 sequences)

SEQ ID NO: 1 - DNA, 21 bp, Artificial sequence
  Primer
agaccaatcctgtcacctctg

SEQ ID NO: 2 - DNA, 19 bp, Artificial sequence
  Primer
cgtctacgctgcagtcctc

SEQ ID NO: 3 - DNA, 22 bp, Artificial sequence
  Primer
gcgctactatactgtctcatgg

SEQ ID NO: 4 - DNA, 21 bp, Artificial sequence
  Primer
ttgtttctcgcataaagcaca

SEQ ID NO: 5 - DNA, 25 bp, Artificial sequence
  Primer
caaagaatgctattagaaaagtgtg

SEQ ID NO: 6 - DNA, 21 bp, Artificial sequence
  Primer
cgacattcatcattatgcctt

SEQ ID NO: 7 - DNA, 23 bp, Artificial sequence
  Primer
accaggaactaatcagacaagga

SEQ ID NO: 8 - DNA, 20 bp, Artificial sequence
  Primer
ggtgtgacttccatgccaat

SEQ ID NO: 9 - DNA, 18 bp, Artificial sequence
  Primer
agatttggacctgcgagc

SEQ ID NO: 10 - DNA, 20 bp, Artificial sequence
  Primer
actgaatagccaaggtgagc

SEQ ID NO: 11 - DNA, 21 bp, Artificial sequence
  Probe
ttgtattcacgctcaccgtgc

SEQ ID NO: 12 - DNA, 25 bp, Artificial sequence
  Probe
tcctggaaattattcaatgcaagta

SEQ ID NO: 13 - DNA, 22 bp, Artificial sequence
  Probe
aaattatggtgatagtgcaaca

SEQ ID NO: 14 - DNA, 20 bp, Artificial sequence
  Probe
cacaatttgcccccagcgct

SEQ ID NO: 15 - DNA, 20 bp, Artificial sequence
  Probe
tccacaagtccgcgcagagc

SEQ ID NO: 16 - DNA, 22 bp, Artificial sequence
  Primer
cgggtgttgctatgcctaatct

SEQ ID NO: 17 - DNA, 22 bp, Artificial sequence
  Primer
ttgcgacattcatcattatgcc

SEQ ID NO: 18 - DNA, 26 bp, Artificial sequence
  Primer
cccaaaattacaatctagtcaagcgt

SEQ ID NO: 19 - DNA, 26 bp, Artificial sequence
  Primer
tgacacagttgagtatattttgcgac

SEQ ID NO: 20 - DNA, 26 bp, Artificial sequence
  Primer
ggccatgtagaaacattttacccaaa

SEQ ID NO: 21 - DNA, 26 bp, Artificial sequence
  Primer
ttgagtatattttgcgacattcatca